European Patent Application EP 4 129 334 A1, published February 8, 2023. Title: Fusion protein suitable for use in disolving fibrin crot and pharamaceutical composition comprising the same. Applicant: National Cancer Center Japan Rin Institute Inc. The sequence listing filed with the application follows.

SEQUENCE LISTING (19 sequences)

SEQ ID NO: 1 - protein, 411 aa, Homo sapiens
SNELHQVPSNCDCLNGGTCVSNKYFSNIHWCNCPKKFGGQHCEIDKSKTCYEGNGHFYRGKASTDTMGRPCLPWNSATVLQQTYHAHRSDALQLGLGKHNYCRNPDNRRRPWCYVQVGLKPLVQECMVHDCADGKKPSSPPEELKFQCGQKTLRPRFKIIGGEFTTIENQPWFAAIYRRHRGGSVTYVCGGSLISPCWVISATHCFIDYPKKEDYIVYLGRSRLNSNTQGEMKFEVENLILHKDYSADTLAHHNDIALLKIRSKEGRCAQPSRTIQTICLPSMYNDPQFGTSCEITGFGKENSTDYLYPEQLKMTVVKLISHRECQQPHYYGSEVTTKMLCAADPQWKTDSCQGDSGGPLVCSLQGRMTLTGIVSWGRGCALKDKPGVYTRVSHFLPWIRSHTKEENGLAL

SEQ ID NO: 2 - protein, 411 aa, Artificial Sequence
  Human pro-urokinase mutant K135G, K136G
SNELHQVPSNCDCLNGGTCVSNKYFSNIHWCNCPKKFGGQHCEIDKSKTCYEGNGHFYRGKASTDTMGRPCLPWNSATVLQQTYHAHRSDALQLGLGKHNYCRNPDNRRRPWCYVQVGLKPLVQECMVHDCADGGGPSSPPEELKFQCGQKTLRPRFKIIGGEFTTIENQPWFAAIYRRHRGGSVTYVCGGSLISPCWVISATHCFIDYPKKEDYIVYLGRSRLNSNTQGEMKFEVENLILHKDYSADTLAHHNDIALLKIRSKEGRCAQPSRTIQTICLPSMYNDPQFGTSCEITGFGKENSTDYLYPEQLKMTVVKLISHRECQQPHYYGSEVTTKMLCAADPQWKTDSCQGDSGGPLVCSLQGRMTLTGIVSWGRGCALKDKPGVYTRVSHFLPWIRSHTKEENGLAL

SEQ ID NO: 3 - protein, 675 aa, Artificial Sequence
  Fusion protein of pro-urokinase mutant and Fab region of heavy chain of anti-fibrin antibdoy 1101 clone
MGSTAILALLLAVLQGVCAEVQLVQSGAEVKKPGESLKISCKGSGYSFTSYWMHWVRQMPGKGLEWIGAIYPGNSDTRYSPSFQGQVTISADKSISTAYLQWSSLKASDTAMYYCTRKAHYGNYGFAYWGQGTLVTVSSASTKGPSVFPLAPSSKSTSGGTAALGCLVKDYFPEPVTVSWNSGALTSGVHTFPAVLQSSGLYSLSSVVTVPSSSLGTQTYICNVNHKPSNTKVDKKVEPKSCGSGGGGSGGGGSGGSSSNELHQVPSNCDCLNGGTCVSNKYFSNIHWCNCPKKFGGQHCEIDKSKTCYEGNGHFYRGKASTDTMGRPCLPWNSATVLQQTYHAHRSDALQLGLGKHNYCRNPDNRRRPWCYVQVGLKPLVQECMVHDCADGGGPSSPPEELKFQCGQKTLRPRFKIIGGEFTTIENQPWFAAIYRRHRGGSVTYVCGGSLISPCWVISATHCFIDYPKKEDYIVYLGRSRLNSNTQGEMKFEVENLILHKDYSADTLAHHNDIALLKIRSKEGRCAQPSRTIQTICLPSMYNDPQFGTSCEITGFGKENSTDYLYPEQLKMTVVKLISHRECQQPHYYGSEVTTKMLCAADPQWKTDSCQGDSGGPLVCSLQGRMTLTGIVSWGRGCALKDKPGVYTRVSHFLPWIRSHTKEENGLALSAGGAS

SEQ ID NO: 4 - protein, 236 aa, Artificial Sequence
  Light chain of humanized 1101 clone
MDMRVPAQLLGLLLLWLRGARCDIQMTQSPSSLSASVGDRVTITCRASQHINNWLAWYQQKPGKAPKLLISGATSLQSGVPSRFSGSGSGTDFTLTISSLQPEDFATYYCQQYWSTPLTFGQGTKVEIKRTVAAPSVFIFPPSDEQLKSGTASVVCLLNNFYPREAKVQWKVDNALQSGNSQESVTEQDSKDSTYSLSSTLTLSKADYEKHKVYACEVTHQGLSSPVTKSFNRGEC

SEQ ID NO: 5 - protein, 242 aa, Artificial Sequence
  Fab region of heavy chain of humanized 1101 clone
MGSTAILALLLAVLQGVCAEVQLVQSGAEVKKPGESLKISCKGSGYSFTSYWMHWVRQMPGKGLEWIGAIYPGNSDTRYSPSFQGQVTISADKSISTAYLQWSSLKASDTAMYYCTRKAHYGNYGFAYWGQGTLVTVSSASTKGPSVFPLAPSSKSTSGGTAALGCLVKDYFPEPVTVSWNSGALTSGVHTFPAVLQSSGLYSLSSVVTVPSSSLGTQTYICNVNHKPSNTKVDKKVEPKSC

SEQ ID NO: 6 - DNA, 41 bp, Artificial Sequence
  Primer 1
acttgaattccaccatgggctctacagcaatcctcgctttg

SEQ ID NO: 7 - DNA, 38 bp, Artificial Sequence
  Primer 2
ataaggatcctttacccggagacagggagaggctcttc

SEQ ID NO: 8 - DNA, 32 bp, Artificial Sequence
  Primer 3
gaggctcgagtcttaagtttcaatgcggccag

SEQ ID NO: 9 - DNA, 78 bp, Artificial Sequence
  Primer 4
ataagcggccgctcaatggtggtggtggtgatgatggtgacttgctccgcctgcggaaagcgccagaccattttcttc

SEQ ID NO: 10 - DNA, 102 bp, Artificial Sequence
  Primer 5
gaagagcctctccctgtctccgggtaaaggatccggtggaggtggcagtggtgggggaggctcaggaggctcgagtcttaagtttcaatgcggccagaaaac

SEQ ID NO: 11 - protein, 5 aa, Artificial Sequence
  HCDR1 of humanized 1101 clone
SYWMH

SEQ ID NO: 12 - protein, 17 aa, Artificial Sequence
  HCDR2 of humanized 1101 clone
AIYPGNSDTRYSPSFQG

SEQ ID NO: 13 - protein, 11 aa, Artificial Sequence
  HCDR3 of humanized 1101 clone
KAHYGNYGFAY

SEQ ID NO: 14 - protein, 11 aa, Artificial Sequence
  LCDR1 of humanized 1101 clone
RASQHINNWLA

SEQ ID NO: 15 - protein, 7 aa, Artificial Sequence
  LCDR2 of humanized 1101 clone
GATSLQS

SEQ ID NO: 16 - protein, 9 aa, Artificial Sequence
  LCDR3 of humanized 1101 clone
QQYWSTPLT

SEQ ID NO: 17 - protein, 16 aa, Artificial Sequence
  Fibrinogen Bbeta 231-246
CNIPVVSGKECEEIIR

SEQ ID NO: 18 - protein, 15 aa, Artificial Sequence
  Fibrinogen gamma 232-246
KNWIQYKEGFGHLSP

SEQ ID NO: 19 - protein, 16 aa, Artificial Sequence
  linker used in Examples
GSGGGGSGGGGSGGSS